European Patent Application EP 4 442 263 A1, published October 9, 2024. Title: Composition for preventing or treating lung disease comprising mesenchymal stem cells overexpressing CD47. Applicant: MEDIPOST CO., LTD. Application KR. The sequence listing filed with the application follows.

SEQUENCE LISTING (4 sequences)

SEQ ID NO: 1 - DNA, 20 bp, synthetic construct
  misc_feature 1..20: note = alpha SMA primer
  source 1..20: mol_type = other DNA
ttgcctgatgggcaagtgat

SEQ ID NO: 2 - DNA, 20 bp, synthetic construct
  misc_feature 1..20: note = alpha SMA primer
  source 1..20: mol_type = other DNA
tacatagtggtgccccctga

SEQ ID NO: 3 - DNA, 24 bp, synthetic construct
  misc_feature 1..24: note = MMP-13 primer
  source 1..24: mol_type = other DNA
tcctcttcttgagctggactcatt

SEQ ID NO: 4 - DNA, 20 bp, synthetic construct
  misc_feature 1..20: note = MMP-13 primer
  source 1..20: mol_type = other DNA
cgctctgcaaactggaggtc